European Patent Application EP 4 321 219 A2, published February 14, 2024. Title: ANTIBODIES AGAINST LIF AND USES THEREOF. Applicant: Medimmune Limited. Application IB PCT/IB2017/001677, filed December 18, 2017. The sequence listing filed with the application follows.

SEQUENCE LISTING (98 sequences)

SEQ ID NO: 1 - protein, 10 aa, synthetic construct
GFTFSHAWMH

SEQ ID NO: 2 - protein, 8 aa, synthetic construct
GFTFSHAW

SEQ ID NO: 3 - protein, 5 aa, synthetic construct
HAWMH

SEQ ID NO: 4 - protein, 10 aa, synthetic construct
GFTFSNAWMH

SEQ ID NO: 5 - protein, 8 aa, synthetic construct
GFTFSNAW

SEQ ID NO: 6 - protein, 5 aa, synthetic construct
NAWMH

SEQ ID NO: 7 - protein, 5 aa, synthetic construct
SKFMY

SEQ ID NO: 8 - protein, 5 aa, synthetic construct
SNFIH

SEQ ID NO: 9 - protein, 19 aa, synthetic construct
QIKAKSDDYATYYAESVKG

SEQ ID NO: 10 - protein, 10 aa, synthetic construct
IKAKSDDYAT

SEQ ID NO: 11 - protein, 19 aa, synthetic construct
QIKDKSDNYATYYAESVKG

SEQ ID NO: 12 - protein, 10 aa, synthetic construct
IKDKSDNYAT

SEQ ID NO: 13 - protein, 17 aa, synthetic construct
WIYPGDGDTEYNQKFSE

SEQ ID NO: 14 - protein, 17 aa, synthetic construct
WIYPGDGDIEYNQKFIG

SEQ ID NO: 15 - protein, 9 aa, synthetic construct
TCWEWDLDF

SEQ ID NO: 16 - protein, 7 aa, synthetic construct
WEWDLDF

SEQ ID NO: 17 - protein, 9 aa, synthetic construct
TCWEWYLDF

SEQ ID NO: 18 - protein, 7 aa, synthetic construct
WEWYLDF

SEQ ID NO: 19 - protein, 10 aa, synthetic construct
RDYHSSHFAY

SEQ ID NO: 20 - protein, 8 aa, synthetic construct
HYSSSMDA

SEQ ID NO: 21 - protein, 16 aa, synthetic construct
RSSQSLLDSDGHTYLN

SEQ ID NO: 22 - protein, 11 aa, synthetic construct
QSLLDSDGHTY

SEQ ID NO: 23 - protein, 16 aa, synthetic construct
RSSQSLLHNNGNTYLS

SEQ ID NO: 24 - protein, 16 aa, synthetic construct
RSSQSLVHSNGNTFLS

SEQ ID NO: 25 - protein, 7 aa, synthetic construct
SVSNLES

SEQ ID NO: 26 - skipped

SEQ ID NO: 27 - protein, 7 aa, synthetic construct
QVSNRFS

SEQ ID NO: 28 - protein, 7 aa, synthetic construct
KVSNRFS

SEQ ID NO: 29 - protein, 10 aa, synthetic construct
MQATHAPPYT

SEQ ID NO: 30 - protein, 9 aa, synthetic construct
GQGTQYPYT

SEQ ID NO: 31 - protein, 9 aa, synthetic construct
GQGTQYPFT

SEQ ID NO: 32 - protein, 6 aa, synthetic construct
SGYYWN

SEQ ID NO: 33 - protein, 5 aa, synthetic construct
TAGMQ

SEQ ID NO: 34 - protein, 16 aa, synthetic construct
CISYDGRNNYNPSLKN

SEQ ID NO: 35 - protein, 17 aa, synthetic construct
WINTQSGEPQYVDDFRG

SEQ ID NO: 36 - protein, 15 aa, synthetic construct
RYRYYNYGSYYAVDY

SEQ ID NO: 37 - protein, 12 aa, synthetic construct
WALYSEYDVMDY

SEQ ID NO: 38 - protein, 11 aa, synthetic construct
RASENIDGYLE

SEQ ID NO: 39 - protein, 11 aa, synthetic construct
KASENVDSYVS

SEQ ID NO: 40 - protein, 7 aa, synthetic construct
AATLLAD

SEQ ID NO: 41 - protein, 7 aa, synthetic construct
GASNRYT

SEQ ID NO: 42 - protein, 9 aa, synthetic construct
QHYYNTPLT

SEQ ID NO: 43 - protein, 9 aa, synthetic construct
GQSYRYPPT

SEQ ID NO: 44 - protein, 25 aa, synthetic construct
EVQLVESGGGLVKPGGSLKLSCAAS

SEQ ID NO: 45 - protein, 25 aa, synthetic construct
QVQLQESGGGLVKPGGSLRLSCAAS

SEQ ID NO: 46 - protein, 25 aa, synthetic construct
EVQLVESGGGVVQPGRSLRLSCAAS

SEQ ID NO: 47 - protein, 25 aa, synthetic construct
EVQLMESGGGLVKPGGSLRLSCATS

SEQ ID NO: 48 - protein, 14 aa, synthetic construct
WVRQAPGKGLEWVA

SEQ ID NO: 49 - protein, 14 aa, synthetic construct
WVRQAPGKGLEWVG

SEQ ID NO: 50 - protein, 30 aa, synthetic construct
RFTISRDDSKNTLYLQMNSLKTEDTAVYYC

SEQ ID NO: 51 - protein, 30 aa, synthetic construct
RFSISRDNAKNSLYLQMNSLRVEDTVVYYC

SEQ ID NO: 52 - protein, 30 aa, synthetic construct
RFTISRDDSKSTLFLQMNNLKTEDTAVYYC

SEQ ID NO: 53 - protein, 11 aa, synthetic construct
WGQGTLVTVSS

SEQ ID NO: 54 - protein, 11 aa, synthetic construct
WGQGTMVTVSS

SEQ ID NO: 55 - protein, 11 aa, synthetic construct
WGQGTTVTVSS

SEQ ID NO: 56 - protein, 23 aa, synthetic construct
DVVMTQSPLSLPVTLGQPASISC

SEQ ID NO: 57 - protein, 23 aa, synthetic construct
DIVMTQTPLSSPVTLGQPASISC

SEQ ID NO: 58 - protein, 23 aa, synthetic construct
DIVMTQTPLSLSVTPGQPASISC

SEQ ID NO: 59 - protein, 23 aa, synthetic construct
DVVMTQSPLSQPVTLGQPASISC

SEQ ID NO: 60 - protein, 15 aa, synthetic construct
WFQQRPGQSPRRLIY

SEQ ID NO: 61 - protein, 15 aa, synthetic construct
WLQQRPGQPPRLLIY

SEQ ID NO: 62 - protein, 15 aa, synthetic construct
WLLQKPGQPPQLLIY

SEQ ID NO: 63 - protein, 15 aa, synthetic construct
WLQQRPGQSPRRLIY

SEQ ID NO: 64 - protein, 32 aa, synthetic construct
GVPDRFSGSGSGTDFTLKISRVEAEDVGLYYC

SEQ ID NO: 65 - protein, 32 aa, synthetic construct
GVPDRFSGSGAGTDFTLKISRVEAEDVGVYYC

SEQ ID NO: 66 - protein, 32 aa, synthetic construct
GVPNRFSGSGSGTDFTLKISRVEAEDVGLYYC

SEQ ID NO: 67 - protein, 32 aa, synthetic construct
GVPDRFNGSGSGTDFTLSISRVEAEDVGVYYC

SEQ ID NO: 68 - protein, 10 aa, synthetic construct
FGQGTKLEIK

SEQ ID NO: 69 - protein, 10 aa, synthetic construct
FGGGTKVEIK

SEQ ID NO: 70 - protein, 10 aa, synthetic construct
FGQGTKVEIK

SEQ ID NO: 71 - protein, 118 aa, synthetic construct
EVQLVESGGGLVKPGGSLKLSCAASGFTFSHAWMHWVRQAPGKGLEWVAQIKAKSDDYATYYAESVKGRFTISRDDSKNTLYLQMNSLKTEDTAVYYCTCWEWDLDFWGQGTLVTVSS

SEQ ID NO: 72 - protein, 118 aa, synthetic construct
QVQLQESGGGLVKPGGSLRLSCAASGFTFSHAWMHWVRQAPGKGLEWVGQIKAKSDDYATYYAESVKGRFTISRDDSKNTLYLQMNSLKTEDTAVYYCTCWEWDLDFWGQGTMVTVSS

SEQ ID NO: 73 - protein, 118 aa, synthetic construct
EVQLVESGGGVVQPGRSLRLSCAASGFTFSHAWMHWVRQAPGKGLEWVAQIKAKSDDYATYYAESVKGRFSISRDNAKNSLYLQMNSLRVEDTVVYYCTCWEWDLDFWGQGTTVTVSS

SEQ ID NO: 74 - protein, 118 aa, synthetic construct
EVQLMESGGGLVKPGGSLRLSCATSGFTFSHAWMHWVRQAPGKGLEWVGQIKAKSDDYATYYAESVKGRFTISRDDSKSTLFLQMNNLKTEDTAVYYCTCWEWDLDFWGQGTLVTVSS

SEQ ID NO: 75 - protein, 113 aa, synthetic construct
DVVMTQSPLSLPVTLGQPASISCRSSQSLLDSDGHTYLNWFQQRPGQSPRRLIYSVSNLESGVPDRFSGSGSGTDFTLKISRVEAEDVGLYYCMQATHAPPYTFGQGTKLEIK

SEQ ID NO: 76 - protein, 113 aa, synthetic construct
DIVMTQTPLSSPVTLGQPASISCRSSQSLLDSDGHTYLNWLQQRPGQPPRLLIYSVSNLESGVPDRFSGSGAGTDFTLKISRVEAEDVGVYYCMQATHAPPYTFGQGTKLEIK

SEQ ID NO: 77 - protein, 113 aa, synthetic construct
DIVMTQTPLSLSVTPGQPASISCRSSQSLLDSDGHTYLNWLLQKPGQPPQLLIYSVSNLESGVPNRFSGSGSGTDFTLKISRVEAEDVGLYYCMQATHAPPYTFGGGTKVEIK

SEQ ID NO: 78 - protein, 113 aa, synthetic construct
DVVMTQSPLSQPVTLGQPASISCRSSQSLLDSDGHTYLNWLQQRPGQSPRRLIYSVSNLESGVPDRFNGSGSGTDFTLSISRVEAEDVGVYYCMQATHAPPYTFGQGTKVEIK

SEQ ID NO: 79 - protein, 467 aa, synthetic construct
MGWTLVFLFLLSVTAGVHSEVQLVESGGGLVKPGGSLKLSCAASGFTFSHAWMHWVRQAPGKGLEWVAQIKAKSDDYATYYAESVKGRFTISRDDSKNTLYLQMNSLKTEDTAVYYCTCWEWDLDFWGQGTLVTVSSASTKGPSVFPLAPSSKSTSGGTAALGCLVKDYFPEPVTVSWNSGALTSGVHTFPAVLQSSGLYSLSSVVTVPSSSLGTQTYICNVNHKPSNTKVDKKVEPKSCDKTHTCPPCPAPELLGGPSVFLFPPKPKDTLMISRTPEVTCVVVDVSHEDPEVKFNWYVDGVEVHNAKTKPREEQYNSTYRVVSVLTVLHQDWLNGKEYKCKVSNKALPAPIEKTISKAKGQPREPQVYTLPPSRDELTKNQVSLTCLVKGFYPSDIAVEWESNGQPENNYKTTPPVLDSDGSFFLYSKLTVDKSRWQQGNVFSCSVMHEALHNHYTQKSLSLSPGK

SEQ ID NO: 80 - protein, 467 aa, synthetic construct
MGWTLVFLFLLSVTAGVHSQVQLQESGGGLVKPGGSLRLSCAASGFTFSHAWMHWVRQAPGKGLEWVGQIKAKSDDYATYYAESVKGRFTISRDDSKNTLYLQMNSLKTEDTAVYYCTCWEWDLDFWGQGTMVTVSSASTKGPSVFPLAPSSKSTSGGTAALGCLVKDYFPEPVTVSWNSGALTSGVHTFPAVLQSSGLYSLSSVVTVPSSSLGTQTYICNVNHKPSNTKVDKKVEPKSCDKTHTCPPCPAPELLGGPSVFLFPPKPKDTLMISRTPEVTCVVVDVSHEDPEVKFNWYVDGVEVHNAKTKPREEQYNSTYRVVSVLTVLHQDWLNGKEYKCKVSNKALPAPIEKTISKAKGQPREPQVYTLPPSRDELTKNQVSLTCLVKGFYPSDIAVEWESNGQPENNYKTTPPVLDSDGSFFLYSKLTVDKSRWQQGNVFSCSVMHEALHNHYTQKSLSLSPGK

SEQ ID NO: 81 - protein, 467 aa, synthetic construct
MGWTLVFLFLLSVTAGVHSEVQLVESGGGVVQPGRSLRLSCAASGFTFSHAWMHWVRQAPGKGLEWVAQIKAKSDDYATYYAESVKGRFSISRDNAKNSLYLQMNSLRVEDTVVYYCTCWEWDLDFWGQGTTVTVSSASTKGPSVFPLAPSSKSTSGGTAALGCLVKDYFPEPVTVSWNSGALTSGVHTFPAVLQSSGLYSLSSVVTVPSSSLGTQTYICNVNHKPSNTKVDKKVEPKSCDKTHTCPPCPAPELLGGPSVFLFPPKPKDTLMISRTPEVTCVVVDVSHEDPEVKFNWYVDGVEVHNAKTKPREEQYNSTYRVVSVLTVLHQDWLNGKEYKCKVSNKALPAPIEKTISKAKGQPREPQVYTLPPSRDELTKNQVSLTCLVKGFYPSDIAVEWESNGQPENNYKTTPPVLDSDGSFFLYSKLTVDKSRWQQGNVFSCSVMHEALHNHYTQKSLSLSPGK

SEQ ID NO: 82 - protein, 467 aa, synthetic construct
MGWTLVFLFLLSVTAGVHSEVQLMESGGGLVKPGGSLRLSCATSGFTFSHAWMHWVRQAPGKGLEWVGQIKAKSDDYATYYAESVKGRFTISRDDSKSTLFLQMNNLKTEDTAVYYCTCWEWDLDFWGQGTLVTVSSASTKGPSVFPLAPSSKSTSGGTAALGCLVKDYFPEPVTVSWNSGALTSGVHTFPAVLQSSGLYSLSSVVTVPSSSLGTQTYICNVNHKPSNTKVDKKVEPKSCDKTHTCPPCPAPELLGGPSVFLFPPKPKDTLMISRTPEVTCVVVDVSHEDPEVKFNWYVDGVEVHNAKTKPREEQYNSTYRVVSVLTVLHQDWLNGKEYKCKVSNKALPAPIEKTISKAKGQPREPQVYTLPPSRDELTKNQVSLTCLVKGFYPSDIAVEWESNGQPENNYKTTPPVLDSDGSFFLYSKLTVDKSRWQQGNVFSCSVMHEALHNHYTQKSLSLSPGK

SEQ ID NO: 83 - protein, 240 aa, synthetic construct
MVSSAQFLGLLLLCFQGTRCDVVMTQSPLSLPVTLGQPASISCRSSQSLLDSDGHTYLNWFQQRPGQSPRRLIYSVSNLESGVPDRFSGSGSGTDFTLKISRVEAEDVGLYYCMQATHAPPYTFGQGTKLEIKRTVAAPSVFIFPPSDEQLKSGTASVVCLLNNFYPREAKVQWKVDNALQSGNSQESVTEQDSKDSTYSLSSTLTLSKADYEKHKVYACEVTHQGLSSPVTKSFNRGEC

SEQ ID NO: 84 - protein, 240 aa, synthetic construct
MVSSAQFLGLLLLCFQGTRCDIVMTQTPLSSPVTLGQPASISCRSSQSLLDSDGHTYLNWLQQRPGQPPRLLIYSVSNLESGVPDRFSGSGAGTDFTLKISRVEAEDVGVYYCMQATHAPPYTFGQGTKLEIKRTVAAPSVFIFPPSDEQLKSGTASVVCLLNNFYPREAKVQWKVDNALQSGNSQESVTEQDSKDSTYSLSSTLTLSKADYEKHKVYACEVTHQGLSSPVTKSFNRGEC

SEQ ID NO: 85 - protein, 240 aa, synthetic construct
MVSSAQFLGLLLLCFQGTRCDIVMTQTPLSLSVTPGQPASISCRSSQSLLDSDGHTYLNWLLQKPGQPPQLLIYSVSNLESGVPNRFSGSGSGTDFTLKISRVEAEDVGLYYCMQATHAPPYTFGGGTKVEIKRTVAAPSVFIFPPSDEQLKSGTASVVCLLNNFYPREAKVQWKVDNALQSGNSQESVTEQDSKDSTYSLSSTLTLSKADYEKHKVYACEVTHQGLSSPVTKSFNRGEC

SEQ ID NO: 86 - protein, 240 aa, synthetic construct
MVSSAQFLGLLLLCFQGTRCDVVMTQSPLSQPVTLGQPASISCRSSQSLLDSDGHTYLNWLQQRPGQSPRRLIYSVSNLESGVPDRFSGSGSGTDFTLSISRVEAEDVGVYYCMQATHAPPYTFGQGTKVEIKRTVAAPSVFIFPPSDEQLKSGTASVVCLLNNFYPREAKVQWKVDNALQSGNSQESVTEQDSKDSTYSLSSTLTLSKADYEKHKVYACEVTHQGLSSPVTKSFNRGEC

SEQ ID NO: 87 - protein, 448 aa, synthetic construct
EVQLVESGGGLVKPGGSLKLSCAASGFTFSHAWMHWVRQAPGKGLEWVAQIKAKSDDYATYYAESVKGRFTISRDDSKNTLYLQMNSLKTEDTAVYYCTCWEWDLDFWGQGTLVTVSSASTKGPSVFPLAPSSKSTSGGTAALGCLVKDYFPEPVTVSWNSGALTSGVHTFPAVLQSSGLYSLSSVVTVPSSSLGTQTYICNVNHKPSNTKVDKKVEPKSCDKTHTCPPCPAPELLGGPSVFLFPPKPKDTLMISRTPEVTCVVVDVSHEDPEVKFNWYVDGVEVHNAKTKPREEQYNSTYRVVSVLTVLHQDWLNGKEYKCKVSNKALPAPIEKTISKAKGQPREPQVYTLPPSRDELTKNQVSLTCLVKGFYPSDIAVEWESNGQPENNYKTTPPVLDSDGSFFLYSKLTVDKSRWQQGNVFSCSVMHEALHNHYTQKSLSLSPGK

SEQ ID NO: 88 - protein, 448 aa, synthetic construct
QVQLQESGGGLVKPGGSLRLSCAASGFTFSHAWMHWVRQAPGKGLEWVGQIKAKSDDYATYYAESVKGRFTISRDDSKNTLYLQMNSLKTEDTAVYYCTCWEWDLDFWGQGTMVTVSSASTKGPSVFPLAPSSKSTSGGTAALGCLVKDYFPEPVTVSWNSGALTSGVHTFPAVLQSSGLYSLSSVVTVPSSSLGTQTYICNVNHKPSNTKVDKKVEPKSCDKTHTCPPCPAPELLGGPSVFLFPPKPKDTLMISRTPEVTCVVVDVSHEDPEVKFNWYVDGVEVHNAKTKPREEQYNSTYRVVSVLTVLHQDWLNGKEYKCKVSNKALPAPIEKTISKAKGQPREPQVYTLPPSRDELTKNQVSLTCLVKGFYPSDIAVEWESNGQPENNYKTTPPVLDSDGSFFLYSKLTVDKSRWQQGNVFSCSVMHEALHNHYTQKSLSLSPGK

SEQ ID NO: 89 - protein, 448 aa, synthetic construct
EVQLVESGGGVVQPGRSLRLSCAASGFTFSHAWMHWVRQAPGKGLEWVAQIKAKSDDYATYYAESVKGRFSISRDNAKNSLYLQMNSLRVEDTVVYYCTCWEWDLDFWGQGTTVTVSSASTKGPSVFPLAPSSKSTSGGTAALGCLVKDYFPEPVTVSWNSGALTSGVHTFPAVLQSSGLYSLSSVVTVPSSSLGTQTYICNVNHKPSNTKVDKKVEPKSCDKTHTCPPCPAPELLGGPSVFLFPPKPKDTLMISRTPEVTCVVVDVSHEDPEVKFNWYVDGVEVHNAKTKPREEQYNSTYRVVSVLTVLHQDWLNGKEYKCKVSNKALPAPIEKTISKAKGQPREPQVYTLPPSRDELTKNQVSLTCLVKGFYPSDIAVEWESNGQPENNYKTTPPVLDSDGSFFLYSKLTVDKSRWQQGNVFSCSVMHEALHNHYTQKSLSLSPGK

SEQ ID NO: 90 - protein, 448 aa, synthetic construct
EVQLMESGGGLVKPGGSLRLSCATSGFTFSHAWMHWVRQAPGKGLEWVGQIKAKSDDYATYYAESVKGRFTISRDDSKSTLFLQMNNLKTEDTAVYYCTCWEWDLDFWGQGTLVTVSSASTKGPSVFPLAPSSKSTSGGTAALGCLVKDYFPEPVTVSWNSGALTSGVHTFPAVLQSSGLYSLSSVVTVPSSSLGTQTYICNVNHKPSNTKVDKKVEPKSCDKTHTCPPCPAPELLGGPSVFLFPPKPKDTLMISRTPEVTCVVVDVSHEDPEVKFNWYVDGVEVHNAKTKPREEQYNSTYRVVSVLTVLHQDWLNGKEYKCKVSNKALPAPIEKTISKAKGQPREPQVYTLPPSRDELTKNQVSLTCLVKGFYPSDIAVEWESNGQPENNYKTTPPVLDSDGSFFLYSKLTVDKSRWQQGNVFSCSVMHEALHNHYTQKSLSLSPGK

SEQ ID NO: 91 - protein, 220 aa, synthetic construct
DVVMTQSPLSLPVTLGQPASISCRSSQSLLDSDGHTYLNWFQQRPGQSPRRLIYSVSNLESGVPDRFSGSGSGTDFTLKISRVEAEDVGLYYCMQATHAPPYTFGQGTKLEIKRTVAAPSVFIFPPSDEQLKSGTASVVCLLNNFYPREAKVQWKVDNALQSGNSQESVTEQDSKDSTYSLSSTLTLSKADYEKHKVYACEVTHQGLSSPVTKSFNRGEC

SEQ ID NO: 92 - protein, 220 aa, synthetic construct
DIVMTQTPLSSPVTLGQPASISCRSSQSLLDSDGHTYLNWLQQRPGQPPRLLIYSVSNLESGVPDRFSGSGAGTDFTLKISRVEAEDVGVYYCMQATHAPPYTFGQGTKLEIKRTVAAPSVFIFPPSDEQLKSGTASVVCLLNNFYPREAKVQWKVDNALQSGNSQESVTEQDSKDSTYSLSSTLTLSKADYEKHKVYACEVTHQGLSSPVTKSFNRGEC

SEQ ID NO: 93 - protein, 220 aa, synthetic construct
DIVMTQTPLSLSVTPGQPASISCRSSQSLLDSDGHTYLNWLLQKPGQPPQLLIYSVSNLESGVPNRFSGSGSGTDFTLKISRVEAEDVGLYYCMQATHAPPYTFGGGTKVEIKRTVAAPSVFIFPPSDEQLKSGTASVVCLLNNFYPREAKVQWKVDNALQSGNSQESVTEQDSKDSTYSLSSTLTLSKADYEKHKVYACEVTHQGLSSPVTKSFNRGEC

SEQ ID NO: 94 - protein, 220 aa, synthetic construct
DVVMTQSPLSQPVTLGQPASISCRSSQSLLDSDGHTYLNWLQQRPGQSPRRLIYSVSNLESGVPDRFSGSGSGTDFTLSISRVEAEDVGVYYCMQATHAPPYTFGQGTKVEIKRTVAAPSVFIFPPSDEQLKSGTASVVCLLNNFYPREAKVQWKVDNALQSGNSQESVTEQDSKDSTYSLSSTLTLSKADYEKHKVYACEVTHQGLSSPVTKSFNRGEC

SEQ ID NO: 95 - protein, 9 aa, synthetic construct
TSWEWDLDF

SEQ ID NO: 96 - protein, 118 aa, synthetic construct
QVQLQESGGGLVKPGGSLRLSCAASGFTFSHAWMHWVRQAPGKGLEWVGQIKAKSDDYATYYAESVKGRFTISRDDSKNTLYLQMNSLKTEDTAVYYCTSWEWDLDFWGQGTMVTVSS

SEQ ID NO: 97 - protein, 448 aa, synthetic construct
QVQLQESGGGLVKPGGSLRLSCAASGFTFSHAWMHWVRQAPGKGLEWVGQIKAKSDDYATYYAESVKGRFTISRDDSKNTLYLQMNSLKTEDTAVYYCTSWEWDLDFWGQGTMVTVSSASTKGPSVFPLAPSSKSTSGGTAALGCLVKDYFPEPVTVSWNSGALTSGVHTFPAVLQSSGLYSLSSVVTVPSSSLGTQTYICNVNHKPSNTKVDKKVEPKSCDKTHTCPPCPAPELLGGPSVFLFPPKPKDTLMISRTPEVTCVVVDVSHEDPEVKFNWYVDGVEVHNAKTKPREEQYNSTYRVVSVLTVLHQDWLNGKEYKCKVSNKALPAPIEKTISKAKGQPREPQVYTLPPSREEMTKNQVSLTCLVKGFYPSDIAVEWESNGQPENNYKTTPPVLDSDGSFFLYSKLTVDKSRWQQGNVFSCSVMHEALHNHYTQKSLSLSPGK

SEQ ID NO: 98 - protein, 180 aa, synthetic construct
SPLPITPVNATCAIRHPCHNNLMNQIRSQLAQLNGSANALFILYYTAQGEPFPNNLDKLCGPNVTDFPPFHANGTEKAKLVELYRIVVYLGTSLGNITRDQKILNPSALSLHSKLNATADILRGLLSNVLCRLCSKYHVGHVDVTYGPDTSGKDVFQKKKLGCQLLGKYKQIIAVLAQAF